European Patent Application EP 4 282 874 A1, published November 29, 2023. Title: Peptides for prevention and treatment of fibrosis. Applicant: NIBEC Co., Ltd. Seoul National University Industry Foundation. The sequence listing filed with the application follows.

SEQUENCE LISTING (20 sequences)

SEQ ID NO: 1 - protein, 21 aa, Artificial Sequence
  Synthetic peptide
YGLRSKSKKFRRPDIQYPDAT

SEQ ID NO: 2 - protein, 15 aa, Artificial Sequence
  Synthetic peptide
GKCSTRGRKSSRRKK

SEQ ID NO: 3 - DNA, 22 bp, Artificial Sequence
  Primer
cctggaaagaatggagatgatg

SEQ ID NO: 4 - DNA, 22 bp, Artificial Sequence
  Primer
atccaaaccactgaaacctctg

SEQ ID NO: 5 - DNA, 20 bp, Artificial Sequence
  Primer
gctggctacttctcgctctg

SEQ ID NO: 6 - DNA, 20 bp, Artificial Sequence
  Primer
tccgcataggactgaccaag

SEQ ID NO: 7 - DNA, 20 bp, Artificial Sequence
  Primer
ggtgaaggtcggtgtgaacg

SEQ ID NO: 8 - DNA, 20 bp, Artificial Sequence
  Primer
ctcgctcctggaagatggtg

SEQ ID NO: 9 - DNA, 20 bp, Artificial Sequence
  Primer
aggggttaagcacaacagca

SEQ ID NO: 10 - DNA, 19 bp, Artificial Sequence
  Primer
acgacgttagcccgttctc

SEQ ID NO: 11 - DNA, 20 bp, Artificial Sequence
  Primer
cgcagctcaggaagaatgtg

SEQ ID NO: 12 - DNA, 20 bp, Artificial Sequence
  Primer
tgaagtacactggcatgacg

SEQ ID NO: 13 - DNA, 18 bp, Artificial Sequence
  Primer
tgggaatccgacgaatgg

SEQ ID NO: 14 - DNA, 20 bp, Artificial Sequence
  Primer
tgcagatcggaccggatact

SEQ ID NO: 15 - DNA, 23 bp, Artificial Sequence
  Primer
tgtccattttctccttctctgga

SEQ ID NO: 16 - DNA, 18 bp, Artificial Sequence
  Primer
tgtccgcgtcccactagc

SEQ ID NO: 17 - DNA, 20 bp, Artificial Sequence
  Primer
ggcctagcgagtggttcttc

SEQ ID NO: 18 - DNA, 20 bp, Artificial Sequence
  Primer
gttaggcttccgattggggt

SEQ ID NO: 19 - DNA, 19 bp, Artificial Sequence
  Primer
acatcgctcagacaccatg

SEQ ID NO: 20 - DNA, 22 bp, Artificial Sequence
  Primer
tgtagttgaggtcaatgaaggg